European Patent Application EP 4 782 464 A1, published July 29, 2026. Title: 抗GCC抗体、嵌合抗原受体及其用途. Applicant: 南京传奇生物科技有限公司. The sequence listing filed with the application follows.

SEQUENCE LISTING (75 sequences)

SEQ ID NO: 1 - protein, 5 aa, synthetic construct
  source 1..5: note = 14C2 HCDR1
NYDMS

SEQ ID NO: 2 - protein, 5 aa, synthetic construct
  source 1..5: note = 21E1 HCDR1
SYDMT

SEQ ID NO: 3 - protein, 5 aa, synthetic construct
  source 1..5: note = 22G5 HCDR1
SYAMT

SEQ ID NO: 4 - protein, 5 aa, synthetic construct
  source 1..5: note = 25E2 HCDR1
KHAMG

SEQ ID NO: 5 - protein, 5 aa, synthetic construct
  source 1..5: note = 48D5 HCDR1
SNAIS

SEQ ID NO: 6 - protein, 16 aa, synthetic construct
  source 1..16: note = 14C2 HCDR2
TIEPDGSTWYASWAKG

SEQ ID NO: 7 - protein, 16 aa, synthetic construct
  source 1..16: note = 21E1 HCDR
SIGDDGNTYYATWAKG

SEQ ID NO: 8 - protein, 16 aa, synthetic construct
  source 1..16: note = 22G5 HCDR2
TINTISTAYYANWAKG

SEQ ID NO: 9 - protein, 16 aa, synthetic construct
  source 1..16: note = 25E2 HCDR2
TIYVSTNTAYASWAKG

SEQ ID NO: 10 - protein, 16 aa, synthetic construct
  source 1..16: note = 48D5 HCDR2
YIGTGGKSFYATWTKG

SEQ ID NO: 11 - protein, 12 aa, synthetic construct
  source 1..12: note = 14C2 HCDR3
GAPDYSSNAFNL

SEQ ID NO: 12 - protein, 7 aa, synthetic construct
  source 1..7: note = 21E1 HCDR3
GWSFCKS

SEQ ID NO: 13 - protein, 7 aa, synthetic construct
  source 1..7: note = 22G5 HCDR3
DHGYYDV

SEQ ID NO: 14 - protein, 15 aa, synthetic construct
  source 1..15: note = 25E2 HCDR3
GGGSSYYTGELYFNL

SEQ ID NO: 15 - protein, 7 aa, synthetic construct
  source 1..7: note = 48D5 HCDR3
GNTYLDL

SEQ ID NO: 16 - protein, 11 aa, synthetic construct
  source 1..11: note = 14C2 LCDR1
QASQSISSYLA

SEQ ID NO: 17 - protein, 12 aa, synthetic construct
  source 1..12: note = 21E1 LCDR1
QSSQSVANNNLA

SEQ ID NO: 18 - protein, 13 aa, synthetic construct
  source 1..13: note = 22G5 LCDR1
QASQSVYKNNYLS

SEQ ID NO: 19 - protein, 11 aa, synthetic construct
  source 1..11: note = 25E2 LCDR1
QVSQSIGSWLA

SEQ ID NO: 20 - protein, 13 aa, synthetic construct
  source 1..13: note = 48D5 LCDR1
QSSQSVYGADYLA

SEQ ID NO: 21 - protein, 7 aa, synthetic construct
  source 1..7: note = 14C2 LCDR2
KASTLAS

SEQ ID NO: 22 - protein, 7 aa, synthetic construct
  source 1..7: note = 21E1 LCDR2
KASTLES

SEQ ID NO: 23 - protein, 7 aa, synthetic construct
  source 1..7: note = 22G5 LCDR2
DASTLAS

SEQ ID NO: 24 - protein, 7 aa, synthetic construct
  source 1..7: note = 25E2 LCDR2
SASTLAS

SEQ ID NO: 25 - protein, 7 aa, synthetic construct
  source 1..7: note = 48D5 LCDR2
RASNLAS

SEQ ID NO: 26 - protein, 13 aa, synthetic construct
  source 1..13: note = 14C2 LCDR3
QSTYAASNKLHFA

SEQ ID NO: 27 - protein, 10 aa, synthetic construct
  source 1..10: note = 21E1 LCDR3
QGAYRSGIMA

SEQ ID NO: 28 - protein, 13 aa, synthetic construct
  source 1..13: note = 22G5 LCDR3
LGEFSCSSGDCAA

SEQ ID NO: 29 - protein, 10 aa, synthetic construct
  source 1..10: note = 25E2 LCDR3
QSYSSASTTA

SEQ ID NO: 30 - protein, 12 aa, synthetic construct
  source 1..12: note = 48D5 LCDR3
QGTYISSDWLNP

SEQ ID NO: 31 - protein, 117 aa, synthetic construct
  source 1..117: note = 14C2 VH
QSLEESGGRLVTPGTPLTLTCTASGFSLSNYDMSWVRQAPGKGLEWIGTIEPDGSTWYASWAKGRLTISRTSTTVDLKMTSLTTEDTATYFCVRGAPDYSSNAFNLWGQGTLVTVSS

SEQ ID NO: 32 - protein, 112 aa, synthetic construct
  source 1..112: note = 21E1 VH
QSLEESGGRLVTPGTPLTLTCTVSGIDLSSYDMTWVRQAPGKGLEWIGSIGDDGNTYYATWAKGRFTISKTSTTVHLKMTSLTTEDTATYFCARGWSFCKSWGQGTLVTVSS

SEQ ID NO: 33 - protein, 112 aa, synthetic construct
  source 1..112: note = 22G5 VH
QSVEESGGRLVTPGTPLTLTCTVSGIDLSSYAMTWVRQAPGEGLEWIGTINTISTAYYANWAKGRFTISKTSTTVDLKIASPTTEDTATYFCARDHGYYDVWGQGTLVTVSS

SEQ ID NO: 34 - protein, 121 aa, synthetic construct
  source 1..121: note = 25E2 VH
QSVEESGGRLVTPGTPLTLTCTVSGIDLNKHAMGWVRQAPTKGLEWIGTIYVSTNTAYASWAKGRFTISKTSSTTVDLKMTSLTTEDTATYFCARGGGSSYYTGELYFNLWGQGTLVTVSS

SEQ ID NO: 35 - protein, 112 aa, synthetic construct
  source 1..112: note = 48D5 VH
QSLEESGGRLVKPDETLTITCTVSGIDLSSNAISWVRQAPGEGLEYIGYIGTGGKSFYATWTKGRFTISKTSTTVDLKMTSLTNEDTAMYFCATGNTYLDLWGQGTLVTVSS

SEQ ID NO: 36 - protein, 122 aa, synthetic construct
  source 1..122: note = PF0098 VH
QVQLQQPGAELVKPGASVKLSCKASGYTFTSYWMHWVKQRPGQGLEWIGEIKPSNGLTNYIEKFKNKATLTVDKSATTAYMQLSSLTAEDSAVYYCTRTITTTEGYWFFDVWGAGTTVTVSS

SEQ ID NO: 37 - protein, 111 aa, synthetic construct
  source 1..111: note = 14C2 VL
DVVMTQTPSSVSEPVGGTVTIKCQASQSISSYLAWYQQKPGQPPKLLIYKASTLASGVSSQFRGSGSGTEFTLTISDLECADAATYYCQSTYAASNKLHFAFGGGTDVVVK

SEQ ID NO: 38 - protein, 109 aa, synthetic construct
  source 1..109: note = 21E1 VL
AQVLTQTASPVSAAVGGTVTISCQSSQSVANNNLAWYQQKPGQPPSPLIYKASTLESGVPSRFSGSGSGTQFALTISGVQCDDAATYYCQGAYRSGIMAFGGGTEVVVR

SEQ ID NO: 39 - protein, 113 aa, synthetic construct
  source 1..113: note = 22G5 VL
AQVLTQTPSSVSAAVGGTVTINCQASQSVYKNNYLSWYQQKPGQPPRLLIYDASTLASGVPSRFKGSGSGTQFTLTISGVQCDDAATYYCLGEFSCSSGDCAAFGGGTEVVVK

SEQ ID NO: 40 - protein, 108 aa, synthetic construct
  source 1..108: note = 25E2 VL
AYDMTQTPASVEVAVGGTVSIKCQVSQSIGSWLAWYQQKPGQPPKLLIYSASTLASGVSSRFKGSGSGTEFTLTISDLACVDAATYYCQSYSSASTTAFGGGTEVVVR

SEQ ID NO: 41 - protein, 112 aa, synthetic construct
  source 1..112: note = 48D5 VL
AQVLTQTPSSVSAAVGGTVTINCQSSQSVYGADYLAWYQQKPGQPPKLLIYRASNLASGVPSRFRGSGSGTQFTLTISEVQCDDAATYYCQGTYISSDWLNPFGGGTEVVVK

SEQ ID NO: 42 - protein, 110 aa, synthetic construct
  source 1..110: note = PF0098 VL
DIVLTQSPASLAVSLGQRATISCRASESVDYYGTSLMQWYQQKPGQPPKLLIYAASNVESGVPARFSGSGSGTDFSLNIHPVEEDDIAMYFCQQTRKVYTFGGGTKLEIK

SEQ ID NO: 43 - protein, 243 aa, synthetic construct
  source 1..243: note = 14C2 scFv
DVVMTQTPSSVSEPVGGTVTIKCQASQSISSYLAWYQQKPGQPPKLLIYKASTLASGVSSQFRGSGSGTEFTLTISDLECADAATYYCQSTYAASNKLHFAFGGGTDVVVKGGGGSGGGGSGGGGSQSLEESGGRLVTPGTPLTLTCTASGFSLSNYDMSWVRQAPGKGLEWIGTIEPDGSTWYASWAKGRLTISRTSTTVDLKMTSLTTEDTATYFCVRGAPDYSSNAFNLWGQGTLVTVSS

SEQ ID NO: 44 - protein, 236 aa, synthetic construct
  source 1..236: note = 21E1 scFv
AQVLTQTASPVSAAVGGTVTISCQSSQSVANNNLAWYQQKPGQPPSPLIYKASTLESGVPSRFSGSGSGTQFALTISGVQCDDAATYYCQGAYRSGIMAFGGGTEVVVRGGGGSGGGGSGGGGSQSLEESGGRLVTPGTPLTLTCTVSGIDLSSYDMTWVRQAPGKGLEWIGSIGDDGNTYYATWAKGRFTISKTSTTVHLKMTSLTTEDTATYFCARGWSFCKSWGQGTLVTVSS

SEQ ID NO: 45 - protein, 240 aa, synthetic construct
  source 1..240: note = 22G5 scFv
AQVLTQTPSSVSAAVGGTVTINCQASQSVYKNNYLSWYQQKPGQPPRLLIYDASTLASGVPSRFKGSGSGTQFTLTISGVQCDDAATYYCLGEFSCSSGDCAAFGGGTEVVVKGGGGSGGGGSGGGGSQSVEESGGRLVTPGTPLTLTCTVSGIDLSSYAMTWVRQAPGEGLEWIGTINTISTAYYANWAKGRFTISKTSTTVDLKIASPTTEDTATYFCARDHGYYDVWGQGTLVTVSS

SEQ ID NO: 46 - protein, 244 aa, synthetic construct
  source 1..244: note = 25E2 scFv
AYDMTQTPASVEVAVGGTVSIKCQVSQSIGSWLAWYQQKPGQPPKLLIYSASTLASGVSSRFKGSGSGTEFTLTISDLACVDAATYYCQSYSSASTTAFGGGTEVVVRGGGGSGGGGSGGGGSQSVEESGGRLVTPGTPLTLTCTVSGIDLNKHAMGWVRQAPTKGLEWIGTIYVSTNTAYASWAKGRFTISKTSSTTVDLKMTSLTTEDTATYFCARGGGSSYYTGELYFNLWGQGTLVTVSS

SEQ ID NO: 47 - protein, 239 aa, synthetic construct
  source 1..239: note = 48D5 scFv
AQVLTQTPSSVSAAVGGTVTINCQSSQSVYGADYLAWYQQKPGQPPKLLIYRASNLASGVPSRFRGSGSGTQFTLTISEVQCDDAATYYCQGTYISSDWLNPFGGGTEVVVKGGGGSGGGGSGGGGSQSLEESGGRLVKPDETLTITCTVSGIDLSSNAISWVRQAPGEGLEYIGYIGTGGKSFYATWTKGRFTISKTSTTVDLKMTSLTNEDTAMYFCATGNTYLDLWGQGTLVTVSS

SEQ ID NO: 48 - protein, 250 aa, synthetic construct
  source 1..250: note = PF0098 scFv
DIVLTQSPASLAVSLGQRATISCRASESVDYYGTSLMQWYQQKPGQPPKLLIYAASNVESGVPARFSGSGSGTDFSLNIHPVEEDDIAMYFCQQTRKVYTFGGGTKLEIKGSTSGSGKPGSGEGSTKGQVQLQQPGAELVKPGASVKLSCKASGYTFTSYWMHWVKQRPGQGLEWIGEIKPSNGLTNYIEKFKNKATLTVDKSATTAYMQLSSLTAEDSAVYYCTRTITTTEGYWFFDVWGAGTTVTVSS

SEQ ID NO: 49 - protein, 487 aa, synthetic construct
  source 1..487: note = 14C2 CAR
MALPVTALLLPLALLLHAARPDVVMTQTPSSVSEPVGGTVTIKCQASQSISSYLAWYQQKPGQPPKLLIYKASTLASGVSSQFRGSGSGTEFTLTISDLECADAATYYCQSTYAASNKLHFAFGGGTDVVVKGGGGSGGGGSGGGGSQSLEESGGRLVTPGTPLTLTCTASGFSLSNYDMSWVRQAPGKGLEWIGTIEPDGSTWYASWAKGRLTISRTSTTVDLKMTSLTTEDTATYFCVRGAPDYSSNAFNLWGQGTLVTVSSTTTPAPRPPTPAPTIASQPLSLRPEACRPAAGGAVHTRGLDFACDIYIWAPLAGTCGVLLLSLVITLYCKRGRKKLLYIFKQPFMRPVQTTQEEDGCSCRFPEEEEGGCELRVKFSRSADAPAYQQGQNQLYNELNLGRREEYDVLDKRRGRDPEMGGKPRRKNPQEGLYNELQKDKMAEAYSEIGMKGERRRGKGHDGLYQGLSTATKDTYDALHMQALPPR

SEQ ID NO: 50 - protein, 480 aa, synthetic construct
  source 1..480: note = 21E1 CAR
MALPVTALLLPLALLLHAARPAQVLTQTASPVSAAVGGTVTISCQSSQSVANNNLAWYQQKPGQPPSPLIYKASTLESGVPSRFSGSGSGTQFALTISGVQCDDAATYYCQGAYRSGIMAFGGGTEVVVRGGGGSGGGGSGGGGSQSLEESGGRLVTPGTPLTLTCTVSGIDLSSYDMTWVRQAPGKGLEWIGSIGDDGNTYYATWAKGRFTISKTSTTVHLKMTSLTTEDTATYFCARGWSFCKSWGQGTLVTVSSTTTPAPRPPTPAPTIASQPLSLRPEACRPAAGGAVHTRGLDFACDIYIWAPLAGTCGVLLLSLVITLYCKRGRKKLLYIFKQPFMRPVQTTQEEDGCSCRFPEEEEGGCELRVKFSRSADAPAYQQGQNQLYNELNLGRREEYDVLDKRRGRDPEMGGKPRRKNPQEGLYNELQKDKMAEAYSEIGMKGERRRGKGHDGLYQGLSTATKDTYDALHMQALPPR

SEQ ID NO: 51 - protein, 484 aa, synthetic construct
  source 1..484: note = 22G5 CAR
MALPVTALLLPLALLLHAARPAQVLTQTPSSVSAAVGGTVTINCQASQSVYKNNYLSWYQQKPGQPPRLLIYDASTLASGVPSRFKGSGSGTQFTLTISGVQCDDAATYYCLGEFSCSSGDCAAFGGGTEVVVKGGGGSGGGGSGGGGSQSVEESGGRLVTPGTPLTLTCTVSGIDLSSYAMTWVRQAPGEGLEWIGTINTISTAYYANWAKGRFTISKTSTTVDLKIASPTTEDTATYFCARDHGYYDVWGQGTLVTVSSTTTPAPRPPTPAPTIASQPLSLRPEACRPAAGGAVHTRGLDFACDIYIWAPLAGTCGVLLLSLVITLYCKRGRKKLLYIFKQPFMRPVQTTQEEDGCSCRFPEEEEGGCELRVKFSRSADAPAYQQGQNQLYNELNLGRREEYDVLDKRRGRDPEMGGKPRRKNPQEGLYNELQKDKMAEAYSEIGMKGERRRGKGHDGLYQGLSTATKDTYDALHMQALPPR

SEQ ID NO: 52 - protein, 488 aa, synthetic construct
  source 1..488: note = 25E2 CAR
MALPVTALLLPLALLLHAARPAYDMTQTPASVEVAVGGTVSIKCQVSQSIGSWLAWYQQKPGQPPKLLIYSASTLASGVSSRFKGSGSGTEFTLTISDLACVDAATYYCQSYSSASTTAFGGGTEVVVRGGGGSGGGGSGGGGSQSVEESGGRLVTPGTPLTLTCTVSGIDLNKHAMGWVRQAPTKGLEWIGTIYVSTNTAYASWAKGRFTISKTSSTTVDLKMTSLTTEDTATYFCARGGGSSYYTGELYFNLWGQGTLVTVSSTTTPAPRPPTPAPTIASQPLSLRPEACRPAAGGAVHTRGLDFACDIYIWAPLAGTCGVLLLSLVITLYCKRGRKKLLYIFKQPFMRPVQTTQEEDGCSCRFPEEEEGGCELRVKFSRSADAPAYQQGQNQLYNELNLGRREEYDVLDKRRGRDPEMGGKPRRKNPQEGLYNELQKDKMAEAYSEIGMKGERRRGKGHDGLYQGLSTATKDTYDALHMQALPPR

SEQ ID NO: 53 - protein, 483 aa, synthetic construct
  source 1..483: note = 48D5 CAR
MALPVTALLLPLALLLHAARPAQVLTQTPSSVSAAVGGTVTINCQSSQSVYGADYLAWYQQKPGQPPKLLIYRASNLASGVPSRFRGSGSGTQFTLTISEVQCDDAATYYCQGTYISSDWLNPFGGGTEVVVKGGGGSGGGGSGGGGSQSLEESGGRLVKPDETLTITCTVSGIDLSSNAISWVRQAPGEGLEYIGYIGTGGKSFYATWTKGRFTISKTSTTVDLKMTSLTNEDTAMYFCATGNTYLDLWGQGTLVTVSSTTTPAPRPPTPAPTIASQPLSLRPEACRPAAGGAVHTRGLDFACDIYIWAPLAGTCGVLLLSLVITLYCKRGRKKLLYIFKQPFMRPVQTTQEEDGCSCRFPEEEEGGCELRVKFSRSADAPAYQQGQNQLYNELNLGRREEYDVLDKRRGRDPEMGGKPRRKNPQEGLYNELQKDKMAEAYSEIGMKGERRRGKGHDGLYQGLSTATKDTYDALHMQALPPR

SEQ ID NO: 54 - protein, 494 aa, synthetic construct
  source 1..494: note = PF0098 CAR
MALPVTALLLPLALLLHAARPDIVLTQSPASLAVSLGQRATISCRASESVDYYGTSLMQWYQQKPGQPPKLLIYAASNVESGVPARFSGSGSGTDFSLNIHPVEEDDIAMYFCQQTRKVYTFGGGTKLEIKGSTSGSGKPGSGEGSTKGQVQLQQPGAELVKPGASVKLSCKASGYTFTSYWMHWVKQRPGQGLEWIGEIKPSNGLTNYIEKFKNKATLTVDKSATTAYMQLSSLTAEDSAVYYCTRTITTTEGYWFFDVWGAGTTVTVSSTTTPAPRPPTPAPTIASQPLSLRPEACRPAAGGAVHTRGLDFACDIYIWAPLAGTCGVLLLSLVITLYCKRGRKKLLYIFKQPFMRPVQTTQEEDGCSCRFPEEEEGGCELRVKFSRSADAPAYQQGQNQLYNELNLGRREEYDVLDKRRGRDPEMGGKPRRKNPQEGLYNELQKDKMAEAYSEIGMKGERRRGKGHDGLYQGLSTATKDTYDALHMQALPPR

SEQ ID NO: 55 - protein, 323 aa, synthetic construct
  source 1..323: note = Rabbit IgG CH1-CH2-CH3
GQPKAPSVFPLAPCCGDTPSSTVTLGCLVKGYLPEPVTVTWNSGTLTNGVRTFPSVRQSSGLYSLSSVVSVTSSSQPVTCNVAHPATNTKVDKTVAPSTCSKPTCPPPELLGGPSVFIFPPKPKDTLMISRTPEVTCVVVDVSQDDPEVQFTWYINNEQVRTARPPLREQQFNSTIRVVSTLPIAHQDWLRGKEFKCKVHNKALPAPIEKTISKARGQPLEPKVYTMGPPREELSSRSVSLTCMINGFYPSDISVEWEKNGKAEDNYKTTPAVLDSDGSYFLYSKLSVPTSEWQRGDVFTCSVMHEALHNHYTQKSISRSPGK

SEQ ID NO: 56 - protein, 104 aa, synthetic construct
  source 1..104: note = Rabbit IgG CL
GDPVAPTVLIFPPAADQVATGTVTIVCVANKYFPDVTVTWEVDGTTQTTGIENSKTPQNSADCTYNLSSTLTLTSTQYNSHKEYTCKVTQGTTSVVQSFNRGDC

SEQ ID NO: 57 - protein, 454 aa, synthetic construct
  source 1..454: note = 22G5 VH-Rabbit IgG CH1-CH2-CH3
MGWSCIILFLVATATGVHSQSVEESGGRLVTPGTPLTLTCTVSGIDLSSYAMTWVRQAPGEGLEWIGTINTISTAYYANWAKGRFTISKTSTTVDLKIASPTTEDTATYFCARDHGYYDVWGQGTLVTVSSGQPKAPSVFPLAPCCGDTPSSTVTLGCLVKGYLPEPVTVTWNSGTLTNGVRTFPSVRQSSGLYSLSSVVSVTSSSQPVTCNVAHPATNTKVDKTVAPSTCSKPTCPPPELLGGPSVFIFPPKPKDTLMISRTPEVTCVVVDVSQDDPEVQFTWYINNEQVRTARPPLREQQFNSTIRVVSTLPIAHQDWLRGKEFKCKVHNKALPAPIEKTISKARGQPLEPKVYTMGPPREELSSRSVSLTCMINGFYPSDISVEWEKNGKAEDNYKTTPAVLDSDGSYFLYSKLSVPTSEWQRGDVFTCSVMHEALHNHYTQKSISRSPGK

SEQ ID NO: 58 - protein, 236 aa, synthetic construct
  source 1..236: note = 22G5 VL- Rabbit IgG CL
MGWSCIILFLVATATGVHSAQVLTQTPSSVSAAVGGTVTINCQASQSVYKNNYLSWYQQKPGQPPRLLIYDASTLASGVPSRFKGSGSGTQFTLTISGVQCDDAATYYCLGEFSCSSGDCAAFGGGTEVVVKGDPVAPTVLIFPPAADQVATGTVTIVCVANKYFPDVTVTWEVDGTTQTTGIENSKTPQNSADCTYNLSSTLTLTSTQYNSHKEYTCKVTQGTTSVVQSFNRGDC

SEQ ID NO: 59 - protein, 464 aa, synthetic construct
  source 1..464: note = PF0098 VH- Rabbit IgG CH1-CH2-CH3
MGWSCIILFLVATATGVHSQVQLQQPGAELVKPGASVKLSCKASGYTFTSYWMHWVKQRPGQGLEWIGEIKPSNGLTNYIEKFKNKATLTVDKSATTAYMQLSSLTAEDSAVYYCTRTITTTEGYWFFDVWGAGTTVTVSSGQPKAPSVFPLAPCCGDTPSSTVTLGCLVKGYLPEPVTVTWNSGTLTNGVRTFPSVRQSSGLYSLSSVVSVTSSSQPVTCNVAHPATNTKVDKTVAPSTCSKPTCPPPELLGGPSVFIFPPKPKDTLMISRTPEVTCVVVDVSQDDPEVQFTWYINNEQVRTARPPLREQQFNSTIRVVSTLPIAHQDWLRGKEFKCKVHNKALPAPIEKTISKARGQPLEPKVYTMGPPREELSSRSVSLTCMINGFYPSDISVEWEKNGKAEDNYKTTPAVLDSDGSYFLYSKLSVPTSEWQRGDVFTCSVMHEALHNHYTQKSISRSPGK

SEQ ID NO: 60 - protein, 233 aa, synthetic construct
  source 1..233: note = PF0098 VL- Rabbit IgG CL
MGWSCIILFLVATATGVHSDIVLTQSPASLAVSLGQRATISCRASESVDYYGTSLMQWYQQKPGQPPKLLIYAASNVESGVPARFSGSGSGTDFSLNIHPVEEDDIAMYFCQQTRKVYTFGGGTKLEIKGDPVAPTVLIFPPAADQVATGTVTIVCVANKYFPDVTVTWEVDGTTQTTGIENSKTPQNSADCTYNLSSTLTLTSTQYNSHKEYTCKVTQGTTSVVQSFNRGDC

SEQ ID NO: 61 - protein, 21 aa, synthetic construct
  source 1..21: note = CD8alpha signal peptide
MALPVTALLLPLALLLHAARP

SEQ ID NO: 62 - protein, 45 aa, synthetic construct
  source 1..45: note = CD8alpha hinge region
TTTPAPRPPTPAPTIASQPLSLRPEACRPAAGGAVHTRGLDFACD

SEQ ID NO: 63 - protein, 24 aa, synthetic construct
  source 1..24: note = CD8alpha transmembrane domain
IYIWAPLAGTCGVLLLSLVITLYC

SEQ ID NO: 64 - protein, 42 aa, synthetic construct
  source 1..42: note = CD137 co-stimulatory signal domain
KRGRKKLLYIFKQPFMRPVQTTQEEDGCSCRFPEEEEGGCEL

SEQ ID NO: 65 - protein, 112 aa, synthetic construct
  source 1..112: note = CD8zeta intracellular signaling domain
RVKFSRSADAPAYQQGQNQLYNELNLGRREEYDVLDKRRGRDPEMGGKPRRKNPQEGLYNELQKDKMAEAYSEIGMKGERRRGKGHDGLYQGLSTATKDTYDALHMQALPPR

SEQ ID NO: 66 - skipped

SEQ ID NO: 67 - protein, 15 aa, synthetic construct
  source 1..15: note = linker 1
GGGGSGGGGSGGGGS

SEQ ID NO: 68 - protein, 17 aa, synthetic construct
  source 1..17: note = linker 2
GSTSGSGKPGSGEGSTK

SEQ ID NO: 69 - protein, 5 aa, synthetic construct
  source 1..5: note = repeat unit of linker
GGGGS

SEQ ID NO: 70 - protein, 20 aa, synthetic construct
  source 1..20: note = linker
GGGGSGGGGSGGGGSGGGGS

SEQ ID NO: 71 - protein, 466 aa, synthetic construct
  source 1..466: note = 14C2 CAR-without signal peptide
DVVMTQTPSSVSEPVGGTVTIKCQASQSISSYLAWYQQKPGQPPKLLIYKASTLASGVSSQFRGSGSGTEFTLTISDLECADAATYYCQSTYAASNKLHFAFGGGTDVVVKGGGGSGGGGSGGGGSQSLEESGGRLVTPGTPLTLTCTASGFSLSNYDMSWVRQAPGKGLEWIGTIEPDGSTWYASWAKGRLTISRTSTTVDLKMTSLTTEDTATYFCVRGAPDYSSNAFNLWGQGTLVTVSSTTTPAPRPPTPAPTIASQPLSLRPEACRPAAGGAVHTRGLDFACDIYIWAPLAGTCGVLLLSLVITLYCKRGRKKLLYIFKQPFMRPVQTTQEEDGCSCRFPEEEEGGCELRVKFSRSADAPAYQQGQNQLYNELNLGRREEYDVLDKRRGRDPEMGGKPRRKNPQEGLYNELQKDKMAEAYSEIGMKGERRRGKGHDGLYQGLSTATKDTYDALHMQALPPR

SEQ ID NO: 72 - protein, 459 aa, synthetic construct
  source 1..459: note = 21E1 CAR-without signal peptide
AQVLTQTASPVSAAVGGTVTISCQSSQSVANNNLAWYQQKPGQPPSPLIYKASTLESGVPSRFSGSGSGTQFALTISGVQCDDAATYYCQGAYRSGIMAFGGGTEVVVRGGGGSGGGGSGGGGSQSLEESGGRLVTPGTPLTLTCTVSGIDLSSYDMTWVRQAPGKGLEWIGSIGDDGNTYYATWAKGRFTISKTSTTVHLKMTSLTTEDTATYFCARGWSFCKSWGQGTLVTVSSTTTPAPRPPTPAPTIASQPLSLRPEACRPAAGGAVHTRGLDFACDIYIWAPLAGTCGVLLLSLVITLYCKRGRKKLLYIFKQPFMRPVQTTQEEDGCSCRFPEEEEGGCELRVKFSRSADAPAYQQGQNQLYNELNLGRREEYDVLDKRRGRDPEMGGKPRRKNPQEGLYNELQKDKMAEAYSEIGMKGERRRGKGHDGLYQGLSTATKDTYDALHMQALPPR

SEQ ID NO: 73 - protein, 463 aa, synthetic construct
  source 1..463: note = 22G5 CAR-without signal peptide
AQVLTQTPSSVSAAVGGTVTINCQASQSVYKNNYLSWYQQKPGQPPRLLIYDASTLASGVPSRFKGSGSGTQFTLTISGVQCDDAATYYCLGEFSCSSGDCAAFGGGTEVVVKGGGGSGGGGSGGGGSQSVEESGGRLVTPGTPLTLTCTVSGIDLSSYAMTWVRQAPGEGLEWIGTINTISTAYYANWAKGRFTISKTSTTVDLKIASPTTEDTATYFCARDHGYYDVWGQGTLVTVSSTTTPAPRPPTPAPTIASQPLSLRPEACRPAAGGAVHTRGLDFACDIYIWAPLAGTCGVLLLSLVITLYCKRGRKKLLYIFKQPFMRPVQTTQEEDGCSCRFPEEEEGGCELRVKFSRSADAPAYQQGQNQLYNELNLGRREEYDVLDKRRGRDPEMGGKPRRKNPQEGLYNELQKDKMAEAYSEIGMKGERRRGKGHDGLYQGLSTATKDTYDALHMQALPPR

SEQ ID NO: 74 - protein, 467 aa, synthetic construct
  source 1..467: note = 25E2 CAR-without signal peptide
AYDMTQTPASVEVAVGGTVSIKCQVSQSIGSWLAWYQQKPGQPPKLLIYSASTLASGVSSRFKGSGSGTEFTLTISDLACVDAATYYCQSYSSASTTAFGGGTEVVVRGGGGSGGGGSGGGGSQSVEESGGRLVTPGTPLTLTCTVSGIDLNKHAMGWVRQAPTKGLEWIGTIYVSTNTAYASWAKGRFTISKTSSTTVDLKMTSLTTEDTATYFCARGGGSSYYTGELYFNLWGQGTLVTVSSTTTPAPRPPTPAPTIASQPLSLRPEACRPAAGGAVHTRGLDFACDIYIWAPLAGTCGVLLLSLVITLYCKRGRKKLLYIFKQPFMRPVQTTQEEDGCSCRFPEEEEGGCELRVKFSRSADAPAYQQGQNQLYNELNLGRREEYDVLDKRRGRDPEMGGKPRRKNPQEGLYNELQKDKMAEAYSEIGMKGERRRGKGHDGLYQGLSTATKDTYDALHMQALPPR

SEQ ID NO: 75 - protein, 462 aa, synthetic construct
  source 1..462: note = 48D5 CAR-without signal peptide
AQVLTQTPSSVSAAVGGTVTINCQSSQSVYGADYLAWYQQKPGQPPKLLIYRASNLASGVPSRFRGSGSGTQFTLTISEVQCDDAATYYCQGTYISSDWLNPFGGGTEVVVKGGGGSGGGGSGGGGSQSLEESGGRLVKPDETLTITCTVSGIDLSSNAISWVRQAPGEGLEYIGYIGTGGKSFYATWTKGRFTISKTSTTVDLKMTSLTNEDTAMYFCATGNTYLDLWGQGTLVTVSSTTTPAPRPPTPAPTIASQPLSLRPEACRPAAGGAVHTRGLDFACDIYIWAPLAGTCGVLLLSLVITLYCKRGRKKLLYIFKQPFMRPVQTTQEEDGCSCRFPEEEEGGCELRVKFSRSADAPAYQQGQNQLYNELNLGRREEYDVLDKRRGRDPEMGGKPRRKNPQEGLYNELQKDKMAEAYSEIGMKGERRRGKGHDGLYQGLSTATKDTYDALHMQALPPR